European Patent Specification EP 3 551 216 B1, published July 10, 2024. Title: METHODS AND MATERIALS FOR USING FIBRIN SUPPORTS FOR RETINAL PIGMENT EPITHELIUM TRANSPLANTATION. Applicant: Mayo Foundation for Medical Education and Research. The sequence listing filed with the application follows.

SEQUENCE LISTING (76 sequences)

SEQ ID NO: 1 - DNA, 20 bp, Artificial
  synthetic oligonucleotide
aacttgggtttggcaagagc

SEQ ID NO: 2 - DNA, 23 bp, Artificial
  synthetic oligonucleoti
ccacactcagaactacaccatca

SEQ ID NO: 3 - DNA, 24 bp, Artificial
  synthetic oligonucleotide
atttataggctggccctcacggaa

SEQ ID NO: 4 - DNA, 24 bp, Artificial
  synthetic oligonucleotide
tgttctgccggagtcataaagcct

SEQ ID NO: 5 - DNA, 20 bp, Artificial
  synthetic oligonucleotide
tgccagagatccccgaaaat

SEQ ID NO: 6 - DNA, 21 bp, Artificial
  synthetic oligonucleotide
ggaatgtgcttcatccctgtt

SEQ ID NO: 7 - DNA, 22 bp, Artificial
  synthetic oligonucleotide
actgcctggatgaactgtatga

SEQ ID NO: 8 - DNA, 20 bp, Artificial
  synthetic oligonucleotide
gagctctccagcaactgtgt

SEQ ID NO: 9 - DNA, 20 bp, Artificial
  synthetic oligonucleotide
tggtctccaacaagcgtctc

SEQ ID NO: 10 - DNA, 21 bp, Artificial
  synthetic oligonucleotide
tcacaaaacttgtcggactgg

SEQ ID NO: 11 - DNA, 23 bp, Artificial
  synthetic oligonucleotide
ccttcctcaccaagtacctgaaa

SEQ ID NO: 12 - DNA, 20 bp, Artificial
  synthetic oligonucleotide
ctcttgctggaaggctggat

SEQ ID NO: 13 - DNA, 21 bp, Artificial
  synthetic oligonucleotide
aagctgcttgagagggtcttt

SEQ ID NO: 14 - DNA, 20 bp, Artificial
  synthetic oligonucleotide
acggccttgccatcatactt

SEQ ID NO: 15 - DNA, 20 bp, Artificial
  synthetic oligonucleotide
ccagggttcaggtttggttc

SEQ ID NO: 16 - DNA, 20 bp, Artificial
  synthetic oligonucleotide
catctgtggagggtcttggg

SEQ ID NO: 17 - DNA, 24 bp, Artificial
  synthetic oligonucleotide
aatacaggaacttgaaatgcaggc

SEQ ID NO: 18 - DNA, 20 bp, Artificial
  synthetic oligonucleotide
atgctgaaggaggtcttggc

SEQ ID NO: 19 - DNA, 20 bp, Artificial
  synthetic oligonucleotide
cgggagatctctgagaccga

SEQ ID NO: 20 - DNA, 20 bp, Artificial
  synthetic oligonucleotide
ggatgagagtgcccagttcc

SEQ ID NO: 21 - DNA, 20 bp, Artificial
  synthetic oligonucleotide
cgcatcaaggagttgggaat

SEQ ID NO: 22 - DNA, 17 bp, Artificial
  synthetic oligonucleotide
ctccaggcggcgagagt

SEQ ID NO: 23 - DNA, 20 bp, Artificial
  synthetic oligonucleotide
ctgctcatcggctgttggta

SEQ ID NO: 24 - DNA, 20 bp, Artificial
  synthetic oligonucleotide
gagcattgggaaccacaggt

SEQ ID NO: 25 - DNA, 21 bp, Artificial
  synthetic oligonucleotide
tgcctgggattcttctcacag

SEQ ID NO: 26 - DNA, 22 bp, Artificial
  synthetic oligonucleotide
tgcttcataagtctgcgcctat

SEQ ID NO: 27 - DNA, 24 bp, Artificial
  synthetic oligonucleotide
ttgacagtatttttgagcagtggc

SEQ ID NO: 28 - DNA, 20 bp, Artificial
  synthetic oligonucleotide
gacacagcaagctcacaagc

SEQ ID NO: 29 - DNA, 21 bp, Artificial
  synthetic oligonucleotide
tctgaaggttctgatgccagc

SEQ ID NO: 30 - DNA, 20 bp, Artificial
  synthetic oligonucleotide
gctggtgatgagagcaaggt

SEQ ID NO: 31 - DNA, 20 bp, Artificial
  synthetic oligonucleotide
aagcaagtgaagggatctgc

SEQ ID NO: 32 - DNA, 20 bp, Artificial
  synthetic oligonucleotide
tcacagaggtttggcttccg

SEQ ID NO: 33 - DNA, 20 bp, Artificial
  synthetic oligonucleotide
cgctctaagggttctgctct

SEQ ID NO: 34 - DNA, 21 bp, Artificial
  synthetic oligonucleotide
tcctgggcagacaccttctta

SEQ ID NO: 35 - DNA, 22 bp, Artificial
  synthetic oligonucleotide
atcctgcttatccttgtgctga

SEQ ID NO: 36 - DNA, 20 bp, Artificial
  synthetic oligonucleotide
gggtcattgtcagccgcttt

SEQ ID NO: 37 - DNA, 20 bp, Artificial
  synthetic oligonucleotide
ggtggacaccatcgtgaaag

SEQ ID NO: 38 - DNA, 20 bp, Artificial
  synthetic oligonucleotide
gaagccatttcatagcgggc

SEQ ID NO: 39 - DNA, 20 bp, Artificial
  synthetic oligonucleotide
aatgtcacctggggcattca

SEQ ID NO: 40 - DNA, 25 bp, Artificial
  synthetic oligonucleotide
aaaagcccatcctgtacattacaaa

SEQ ID NO: 41 - DNA, 21 bp, Artificial
  synthetic oligonucleotide
cttcaaggggcagtgggtaac

SEQ ID NO: 42 - DNA, 20 bp, Artificial
  synthetic oligonucleotide
ggacttggtgacttcgcctt

SEQ ID NO: 43 - DNA, 20 bp, Artificial
  synthetic oligonucleotide
tccgaaccaagcttcgtatc

SEQ ID NO: 44 - DNA, 20 bp, Artificial
  synthetic oligonucleotide
tagcgaaagtgccaaagctg

SEQ ID NO: 45 - DNA, 20 bp, Artificial
  synthetic oligonucleotide
tggacacctcctggctattg

SEQ ID NO: 46 - DNA, 20 bp, Artificial
  synthetic oligonucleotide
gggccaggatgaagtcgtag

SEQ ID NO: 47 - DNA, 20 bp, Artificial
  synthetic oligonucleotide
ctgcagttcgaggtgctcat

SEQ ID NO: 48 - DNA, 15 bp, Artificial
  synthetic oligonucleotide
aggcggccggcagag

SEQ ID NO: 49 - DNA, 20 bp, Artificial
  synthetic oligonucleotide
accacttttaggtcggctca

SEQ ID NO: 50 - DNA, 20 bp, Artificial
  synthetic oligonucleotide
tctggtccggagattctgct

SEQ ID NO: 51 - DNA, 21 bp, Artificial
  synthetic oligonucleotide
aactcttcctgaggcaggtgg

SEQ ID NO: 52 - DNA, 20 bp, Artificial
  synthetic oligonucleotide
ggaatctacggggtgggttt

SEQ ID NO: 53 - DNA, 20 bp, Artificial
  synthetic oligonucleotide
gccagacgatcatgcagcta

SEQ ID NO: 54 - DNA, 24 bp, Artificial
  synthetic oligonucleotide
gcagtctacatgctaaatcagagg

SEQ ID NO: 55 - DNA, 20 bp, Artificial
  synthetic oligonucleotide
tcgagggtgcaggtatggtt

SEQ ID NO: 56 - DNA, 20 bp, Artificial
  synthetic oligonucleotide
tctgaactcacttcccgagc

SEQ ID NO: 57 - DNA, 23 bp, Artificial
  synthetic oligonucleotide
gatcaagatcattgctcctcctg

SEQ ID NO: 58 - DNA, 22 bp, Artificial
  synthetic oligonucleotide
ctgcgcaagttaggttttgtca

SEQ ID NO: 59 - DNA, 20 bp, Artificial
  synthetic oligonucleotide
ctctgctcctcctgttcgac

SEQ ID NO: 60 - DNA, 20 bp, Artificial
  synthetic oligonucleotide
accaaatccgttgactccga

SEQ ID NO: 61 - DNA, 22 bp, Artificial
  synthetic oligonucleotide
agatcaaaaggagacaggtgct

SEQ ID NO: 62 - DNA, 20 bp, Artificial
  synthetic oligonucleotide
aatagcccccacccattgtg

SEQ ID NO: 63 - DNA, 19 bp, Artificial
  synthetic oligonucleotide
actgacggagcccgagaag

SEQ ID NO: 64 - DNA, 20 bp, Artificial
  synthetic oligonucleotide
ttgctcggttctcttcaccc

SEQ ID NO: 65 - DNA, 22 bp, Artificial
  synthetic oligonucleotide
ttggcttaatgagactgggacc

SEQ ID NO: 66 - DNA, 21 bp, Artificial
  synthetic oligonucleotide
acatcaccacaccaacactga

SEQ ID NO: 67 - DNA, 18 bp, Artificial
  synthetic oligonucleotide
gtgacgcagaaggcctca

SEQ ID NO: 68 - DNA, 20 bp, Artificial
  synthetic oligonucleotide
tgcaccaggtctgagtgttc

SEQ ID NO: 69 - DNA, 22 bp, Artificial
  synthetic oligonucleotide
ggatcactaggtgatatcgagc

SEQ ID NO: 70 - DNA, 29 bp, Artificial
  synthetic oligonucleotide
accagacaagagtttaagagatatgtatc

SEQ ID NO: 71 - DNA, 22 bp, Artificial
  synthetic oligonucleotide
ttcctgcatgccagaggagccc

SEQ ID NO: 72 - DNA, 20 bp, Artificial
  synthetic oligonucleotide
aatgtatcgaaggtgctcaa

SEQ ID NO: 73 - DNA, 23 bp, Artificial
  synthetic oligonucleotide
atgcaccgctacgacgtgagcgc

SEQ ID NO: 74 - DNA, 21 bp, Artificial
  synthetic oligonucleotide
accttgacaatcctgatgtgg

SEQ ID NO: 75 - DNA, 22 bp, Artificial
  synthetic oligonucleotide
taactgactagcaggcttgtcg

SEQ ID NO: 76 - DNA, 26 bp, Artificial
  synthetic oligonucleotide
tccacatacagtcctggatgatgatg